European Patent Application EP 4 631 521 A1, published October 15, 2025. Title: CANCER COMBINATION THERAPY USING CD24 ANTIBODY AND PD-1-PD-L1 PATHWAY BLOCKING ANTIBODY. Applicant: ImmuneOnco Biopharmaceuticals (Shanghai) Inc. Application EP EP23899665.6, filed November 1, 2023. The sequence listing filed with the application follows.

SEQUENCE LISTING (19 sequences)

SEQ ID NO: 1 - protein, 9 aa, synthetic construct
GYSITSGYS

SEQ ID NO: 2 - protein, 7 aa, synthetic construct
IHYSGST

SEQ ID NO: 3 - protein, 10 aa, synthetic construct
ARGADYALDY

SEQ ID NO: 4 - protein, 12 aa, synthetic construct
QSLLYSSNQKNY

SEQ ID NO: 5 - protein, 9 aa, synthetic construct
QQNFIYPLT

SEQ ID NO: 6 - protein, 117 aa, synthetic construct
DVQLQESGPDLVKPSQSLSLTCTVTGYSITSGYSWHWIRQFPGNKLEWMGYIHYSGSTKYNPSLKSRISITRDTSKNQFFLQLNSVTTEDTATYFCARGADYALDYWGQRTSVTVSS

SEQ ID NO: 7 - protein, 113 aa, synthetic construct
DIQMTQSPSSLSASVGDRVTITCKSSQSLLYSSNQKNYLAWYQQKPGKAPKLLIYWASTRESGVPSRFSGSGSGTDFTLTISSLQPEDFATYYCQQNFIYPLTFGGGTKVELK

SEQ ID NO: 8 - protein, 330 aa, synthetic construct
ASTKGPSVFPLAPSSKSTSGGTAALGCLVKDYFPEPVTVSWNSGALTSGVHTFPAVLQSSGLYSLSSVVTVPSSSLGTQTYICNVNHKPSNTKVDKRVEPKSCDKTHTCPPCPAPELLGGPSVFLFPPKPKDTLMISRTPEVTCVVVDVSHEDPEVKFNWYVDGVEVHNAKTKPREEQYNATYRVVSVLTVLHQDWLNGKEYKCKVSNKALPAPIAATISKAKGQPREPQVYTLPPSREEMTKNQVSLTCLVKGFYPSDIAVEWESNGQPENNYKTTPPVLDSDGSFFLYSKLTVDKSRWQQGNVFSCSVMHEALHNHYTQKSLSLSPGK

SEQ ID NO: 9 - protein, 107 aa, synthetic construct [sequence omitted]

SEQ ID NO: 10 - protein, 113 aa, synthetic construct
DIVMSQSPSSLAVSVGEKVTMSCKSSQSLLYSSNQKNYLAWYQQKPGHSPKLLIYWASTRESGVPDRFTGSGSGTDFTLTISSVKAEDLAVYYCQQNFIYPLTFGAGTKLELK

SEQ ID NO: 11 - protein, 117 aa, synthetic construct
DVQLQESGPGLVKPSETLSLTCTVSGYSITSGYSWHWIRQPPGKGLEWIGYIHYSGSTKYNPSLKSRVTISVDTSKNQFSLKLSSVTAADTAVYYCARGADYALDYWGQRTSVTVSS

SEQ ID NO: 12 - protein, 113 aa, synthetic construct
DIVMTQSPDSLAVSLGERATINCKSSQSLLYSSNQKNYLAWYQQKPGQPPKLLIYWASTRESGVPDRFSGSGSGTDFTLTISSLQAEDVAVYYCQQNFIYPLTFGGGTKVELK

SEQ ID NO: 13 - protein, 8 aa, synthetic construct
GYTFTSNW

SEQ ID NO: 14 - protein, 8 aa, synthetic construct
IHPNSGSS

SEQ ID NO: 15 - protein, 14 aa, synthetic construct
ARSYYGSSPYYFDY

SEQ ID NO: 16 - protein, 6 aa, synthetic construct
QDIINY

SEQ ID NO: 17 - protein, 9 aa, synthetic construct
QQGDTLPWT

SEQ ID NO: 18 - protein, 121 aa, synthetic construct
QVQLVQSGAEVKKPGASVKVSCKASGYTFTSNWMHWVRQAPGQGLEWMGMIHPNSGSSNYNEKFKSRVTMTRDTSTSTVYMELSSLRSEDTAVYYCARSYYGSSPYYFDYWGQGTLVTVSS

SEQ ID NO: 19 - protein, 107 aa, synthetic construct
DIQMTQSPSSLSASVGDRVTITCRASQDIINYLNWYQQKPGKAPKLLIYYTSRLHSGVPSRFSGSGSGTDFTFTISSLQPEDIATYYCQQGDTLPWTFGQGTKVEIK